European Patent Application EP 4 245 308 A1, published September 20, 2023. Title: Cell preparation for use to suppress loss of muscle mass. Applicant: Human Life CORD Japan Inc. The sequence listing filed with the application follows.

SEQUENCE LISTING (16 sequences)

SEQ ID NO: 1 - DNA, 20 bp, Artificial Sequence
  forward primer of PGC1-alpha
ccgagaattcatggagcaat

SEQ ID NO: 2 - DNA, 20 bp, Artificial Sequence
  reverse primer of PGC1-alpha
tttctgtgggtttggtgtga

SEQ ID NO: 3 - DNA, 20 bp, Artificial Sequence
  forward primer of COX4
agctgagccaagcagagaag

SEQ ID NO: 4 - DNA, 20 bp, Artificial Sequence
  reverse primer of COX4
aatcaccagagccgtgaatc

SEQ ID NO: 5 - DNA, 20 bp, Artificial Sequence
  forward primer of GLUT4
gacggacactccatctgttg

SEQ ID NO: 6 - DNA, 19 bp, Artificial Sequence
  reverse primer of GLUT4
gccacgatggagacatagc

SEQ ID NO: 7 - DNA, 21 bp, Artificial Sequence
  forward primer of GAPDH
atgtgtccgtcgtggatctga

SEQ ID NO: 8 - DNA, 21 bp, Artificial Sequence
  reverse primer of GAPDH
atgcctgcttcaccaccttct

SEQ ID NO: 9 - DNA, 23 bp, Artificial Sequence
  forward primer of TNF-alpha
gactttctcctggtatgagatag

SEQ ID NO: 10 - DNA, 18 bp, Artificial Sequence
  reverse primer of TNF-alpha
aggctgccccgactacgt

SEQ ID NO: 11 - DNA, 22 bp, Artificial Sequence
  forward primer of MCP-1
gccccactcacctgctgctact

SEQ ID NO: 12 - DNA, 23 bp, Artificial Sequence
  reverse primer of MCP-1
cctgctgctggtgatcctcttgt

SEQ ID NO: 13 - DNA, 20 bp, Artificial Sequence
  forward primer of TGF-beta1
tggagcaacatgtggaactc

SEQ ID NO: 14 - DNA, 18 bp, Artificial Sequence
  reverse primer of TGF-beta1
gtcagcagccggttacca

SEQ ID NO: 15 - DNA, 21 bp, Artificial Sequence
  forward primer of CatK
agcaggctggaggactaaggt

SEQ ID NO: 16 - DNA, 23 bp, Artificial Sequence
  reverse primer of CatK
tttgtgcatctcagtggaagact